European Patent Application EP 4 477 745 A1, published December 18, 2024. Title: Chemically defined culture system for intestinal stem cells derived from 3D intestinal organoids. Applicant: 한국생명공학연구원. Application KR. The sequence listing filed with the application follows.

SEQUENCE LISTING (92 sequences)

SEQ ID NO: 1 - DNA, 19 bp, synthetic construct
  source 1..19: mol_type = other DNA
gaaggtgaaggtcggagtc

SEQ ID NO: 2 - DNA, 20 bp, synthetic construct
  source 1..20: mol_type = other DNA
gaagatggtgatgggatttc

SEQ ID NO: 3 - DNA, 20 bp, synthetic construct
  source 1..20: mol_type = other DNA
tgctcttcaccaactgcatc

SEQ ID NO: 4 - DNA, 20 bp, synthetic construct
  source 1..20: mol_type = other DNA
ctcaggctcaccagatcctc

SEQ ID NO: 5 - DNA, 22 bp, synthetic construct
  source 1..22: mol_type = other DNA
ccagaaggaacagtggtttggc

SEQ ID NO: 6 - DNA, 22 bp, synthetic construct
  source 1..22: mol_type = other DNA
actgtcctctgggcttggtgtt

SEQ ID NO: 7 - DNA, 19 bp, synthetic construct
  source 1..19: mol_type = other DNA
gtacccgcacttgcacaac

SEQ ID NO: 8 - DNA, 21 bp, synthetic construct
  source 1..21: mol_type = other DNA
tctcgctctcgttcagaagtc

SEQ ID NO: 9 - DNA, 19 bp, synthetic construct
  source 1..19: mol_type = other DNA
gaccctttctgaccgacaa

SEQ ID NO: 10 - DNA, 18 bp, synthetic construct
  source 1..18: mol_type = other DNA
cgctttccacggctcttt

SEQ ID NO: 11 - DNA, 21 bp, synthetic construct
  source 1..21: mol_type = other DNA
aaaaccccaggagcagttaat

SEQ ID NO: 12 - DNA, 20 bp, synthetic construct
  source 1..20: mol_type = other DNA
caaccctctttgcacaagct

SEQ ID NO: 13 - DNA, 22 bp, synthetic construct
  source 1..22: mol_type = other DNA
tgaccctgatgagaaagctcaa

SEQ ID NO: 14 - DNA, 21 bp, synthetic construct
  source 1..21: mol_type = other DNA
ccctgagcaacactgtctttt

SEQ ID NO: 15 - DNA, 22 bp, synthetic construct
  source 1..22: mol_type = other DNA
gagtggacttgtgccgacttca

SEQ ID NO: 16 - DNA, 22 bp, synthetic construct
  source 1..22: mol_type = other DNA
ggtggctggtgcaaagacatag

SEQ ID NO: 17 - DNA, 25 bp, synthetic construct
  source 1..25: mol_type = other DNA
tctgaggacaagccacaagattaca

SEQ ID NO: 18 - DNA, 22 bp, synthetic construct
  source 1..22: mol_type = other DNA
tgggcaccaatatcaagtccaa

SEQ ID NO: 19 - DNA, 20 bp, synthetic construct
  source 1..20: mol_type = other DNA
cgtgaagctggtgaacttgg

SEQ ID NO: 20 - DNA, 20 bp, synthetic construct
  source 1..20: mol_type = other DNA
ggatgtactccacggctgag

SEQ ID NO: 21 - DNA, 20 bp, synthetic construct
  source 1..20: mol_type = other DNA
acctttcccgtggacagagt

SEQ ID NO: 22 - DNA, 23 bp, synthetic construct
  source 1..23: mol_type = other DNA
tggacatattccctcactttgga

SEQ ID NO: 23 - DNA, 20 bp, synthetic construct
  source 1..20: mol_type = other DNA
agccagatcactgctgaggt

SEQ ID NO: 24 - DNA, 20 bp, synthetic construct
  source 1..20: mol_type = other DNA
tggacaggtgttcctccttc

SEQ ID NO: 25 - DNA, 24 bp, synthetic construct
  source 1..24: mol_type = other DNA
gtcactgacaccaacgataatcct

SEQ ID NO: 26 - DNA, 25 bp, synthetic construct
  source 1..25: mol_type = other DNA
tttcagtgtggtgattacgacgtta

SEQ ID NO: 27 - DNA, 22 bp, synthetic construct
  source 1..22: mol_type = other DNA
ggaggaatgtgagctggagaca

SEQ ID NO: 28 - DNA, 22 bp, synthetic construct
  source 1..22: mol_type = other DNA
tatgtcgccgttgagttcggtc

SEQ ID NO: 29 - DNA, 20 bp, synthetic construct
  source 1..20: mol_type = other DNA
tggcctacacaagcatctgg

SEQ ID NO: 30 - DNA, 20 bp, synthetic construct
  source 1..20: mol_type = other DNA
taactggctgctgtaacggg

SEQ ID NO: 31 - DNA, 20 bp, synthetic construct
  source 1..20: mol_type = other DNA
ggcagtctgggagttttagg

SEQ ID NO: 32 - DNA, 20 bp, synthetic construct
  source 1..20: mol_type = other DNA
atgccaaaatgaggcaagtc

SEQ ID NO: 33 - DNA, 20 bp, synthetic construct
  source 1..20: mol_type = other DNA
tgtaggcatcgctcttctca

SEQ ID NO: 34 - DNA, 20 bp, synthetic construct
  source 1..20: mol_type = other DNA
gacaccatctacctcacccg

SEQ ID NO: 35 - DNA, 20 bp, synthetic construct
  source 1..20: mol_type = other DNA
tgacctcaacgatgcatttc

SEQ ID NO: 36 - DNA, 20 bp, synthetic construct
  source 1..20: mol_type = other DNA
ctgtcctggctcttctgctc

SEQ ID NO: 37 - DNA, 22 bp, synthetic construct
  source 1..22: mol_type = other DNA
gaggacctgttcatcgtcagca

SEQ ID NO: 38 - DNA, 22 bp, synthetic construct
  source 1..22: mol_type = other DNA
cgtccagatagctcagcttcag

SEQ ID NO: 39 - DNA, 22 bp, synthetic construct
  source 1..22: mol_type = other DNA
caccagtggttggaaggacatg

SEQ ID NO: 40 - DNA, 22 bp, synthetic construct
  source 1..22: mol_type = other DNA
catcgtccacattccgctcctt

SEQ ID NO: 41 - DNA, 22 bp, synthetic construct
  source 1..22: mol_type = other DNA
gtcaagaaggctctcagacctc

SEQ ID NO: 42 - DNA, 22 bp, synthetic construct
  source 1..22: mol_type = other DNA
gttcatcctcgttgagctggag

SEQ ID NO: 43 - DNA, 23 bp, synthetic construct
  source 1..23: mol_type = other DNA
ccagtggatagagccattgaaga

SEQ ID NO: 44 - DNA, 22 bp, synthetic construct
  source 1..22: mol_type = other DNA
tctcaggagagtggaccacact

SEQ ID NO: 45 - DNA, 22 bp, synthetic construct
  source 1..22: mol_type = other DNA
gggcactgagtgccattacttc

SEQ ID NO: 46 - DNA, 22 bp, synthetic construct
  source 1..22: mol_type = other DNA
cggcattgttcaccaggatggt

SEQ ID NO: 47 - DNA, 22 bp, synthetic construct
  source 1..22: mol_type = other DNA
ggcatcaccttctggaatgtcc

SEQ ID NO: 48 - DNA, 23 bp, synthetic construct
  source 1..23: mol_type = other DNA
ccagcatcgtaggaagaaaagcc

SEQ ID NO: 49 - DNA, 23 bp, synthetic construct
  source 1..23: mol_type = other DNA
cggtatttctggagatagtgcag

SEQ ID NO: 50 - DNA, 22 bp, synthetic construct
  source 1..22: mol_type = other DNA
tcaagaggctgaagggcaggat

SEQ ID NO: 51 - DNA, 22 bp, synthetic construct
  source 1..22: mol_type = other DNA
gctgtcctactgcttggaagac

SEQ ID NO: 52 - DNA, 22 bp, synthetic construct
  source 1..22: mol_type = other DNA
ctgcatcagcacatactcctcc

SEQ ID NO: 53 - DNA, 22 bp, synthetic construct
  source 1..22: mol_type = other DNA
ctgcatcagcacatactcctcc

SEQ ID NO: 54 - DNA, 22 bp, synthetic construct
  source 1..22: mol_type = other DNA
ccaggatttggatgaccagcca

SEQ ID NO: 55 - DNA, 22 bp, synthetic construct
  source 1..22: mol_type = other DNA
ccaggatttggatgaccagcca

SEQ ID NO: 56 - DNA, 22 bp, synthetic construct
  source 1..22: mol_type = other DNA
gtccttggagaggaagccattc

SEQ ID NO: 57 - DNA, 22 bp, synthetic construct
  source 1..22: mol_type = other DNA
cagcgagatgttcccgcaaatc

SEQ ID NO: 58 - DNA, 23 bp, synthetic construct
  source 1..23: mol_type = other DNA
gcctctgtgtagacgatgaatgc

SEQ ID NO: 59 - DNA, 23 bp, synthetic construct
  source 1..23: mol_type = other DNA
gatgctggagtaccttgtgactg

SEQ ID NO: 60 - DNA, 22 bp, synthetic construct
  source 1..22: mol_type = other DNA
caggtgagaaggcacaacagct

SEQ ID NO: 61 - DNA, 20 bp, synthetic construct
  source 1..20: mol_type = other DNA
caaattgaagcagccagaca

SEQ ID NO: 62 - DNA, 20 bp, synthetic construct
  source 1..20: mol_type = other DNA
ggagttgggagacccatgta

SEQ ID NO: 63 - DNA, 20 bp, synthetic construct
  source 1..20: mol_type = other DNA
cctttgcaggaaatggactc

SEQ ID NO: 64 - DNA, 20 bp, synthetic construct
  source 1..20: mol_type = other DNA
ggactcacgggtagcacaac

SEQ ID NO: 65 - DNA, 22 bp, synthetic construct
  source 1..22: mol_type = other DNA
tgtgagtccttcagctgtggaa

SEQ ID NO: 66 - DNA, 19 bp, synthetic construct
  source 1..19: mol_type = other DNA
ggaactcaacacaccattg

SEQ ID NO: 67 - DNA, 20 bp, synthetic construct
  source 1..20: mol_type = other DNA
cattgccatctttgcctgtg

SEQ ID NO: 68 - DNA, 21 bp, synthetic construct
  source 1..21: mol_type = other DNA
agccataaccatagccatagc

SEQ ID NO: 69 - DNA, 20 bp, synthetic construct
  source 1..20: mol_type = other DNA
cccagtcaatgccaggtacg

SEQ ID NO: 70 - DNA, 20 bp, synthetic construct
  source 1..20: mol_type = other DNA
gggccttggtgttgggtaag

SEQ ID NO: 71 - DNA, 20 bp, synthetic construct
  source 1..20: mol_type = other DNA
caggctacgaccgcaaggac

SEQ ID NO: 72 - DNA, 20 bp, synthetic construct
  source 1..20: mol_type = other DNA
ggtggtggtggtggtgttgg

SEQ ID NO: 73 - DNA, 20 bp, synthetic construct
  source 1..20: mol_type = other DNA
gcagcccctgtgaagattga

SEQ ID NO: 74 - DNA, 20 bp, synthetic construct
  source 1..20: mol_type = other DNA
gtctctggcaaaaagcggtg

SEQ ID NO: 75 - DNA, 22 bp, synthetic construct
  source 1..22: mol_type = other DNA
tccattggtcttctgtcacccg

SEQ ID NO: 76 - DNA, 22 bp, synthetic construct
  source 1..22: mol_type = other DNA
agaccatccacctccacttctc

SEQ ID NO: 77 - DNA, 21 bp, synthetic construct
  source 1..21: mol_type = other DNA
gaggatgccctgagacacgga

SEQ ID NO: 78 - DNA, 22 bp, synthetic construct
  source 1..22: mol_type = other DNA
ccagaaaggagtagacgaagcc

SEQ ID NO: 79 - DNA, 19 bp, synthetic construct
  source 1..19: mol_type = other DNA
atggtggtgtcgtgcatct

SEQ ID NO: 80 - DNA, 18 bp, synthetic construct
  source 1..18: mol_type = other DNA
cgctgcagggaggtagag

SEQ ID NO: 81 - DNA, 20 bp, synthetic construct
  source 1..20: mol_type = other DNA
ccacctcattctcctggcta

SEQ ID NO: 82 - DNA, 20 bp, synthetic construct
  source 1..20: mol_type = other DNA
aggtcccatttttcctttcg

SEQ ID NO: 83 - DNA, 18 bp, synthetic construct
  source 1..18: mol_type = other DNA
atcatgtgcgtgctgtcg

SEQ ID NO: 84 - DNA, 21 bp, synthetic construct
  source 1..21: mol_type = other DNA
tgcagtgctcaactgatgtct

SEQ ID NO: 85 - DNA, 18 bp, synthetic construct
  source 1..18: mol_type = other DNA
ctccctggtggtgctcat

SEQ ID NO: 86 - DNA, 22 bp, synthetic construct
  source 1..22: mol_type = other DNA
ggctgatataactggttgacga

SEQ ID NO: 87 - DNA, 20 bp, synthetic construct
  source 1..20: mol_type = other DNA
gaccccaaaatcagcgaaat

SEQ ID NO: 88 - DNA, 24 bp, synthetic construct
  source 1..24: mol_type = other DNA
tctggttactgccagttgaatctg

SEQ ID NO: 89 - DNA, 19 bp, synthetic construct
  source 1..19: mol_type = other DNA
agcagtacgcacacaatcg

SEQ ID NO: 90 - DNA, 22 bp, synthetic construct
  source 1..22: mol_type = other DNA
ttcggaagagacaggtacgtta

SEQ ID NO: 91 - DNA, 20 bp, synthetic construct
  source 1..20: mol_type = other DNA
ctcctctagtggcggctatt

SEQ ID NO: 92 - DNA, 20 bp, synthetic construct
  source 1..20: mol_type = other DNA
agaatagagctcgcaccgta